European Patent Application EP 4 502 159 A1, published February 5, 2025. Title: ENGINEERED IMMUNE CELL WITH CIITA GENE KNOCK-OUT AND USE THEREOF. Applicant: NANJING BIOHENG BIOTECH CO., LTD. Application EP. The sequence listing filed with the application follows.

SEQUENCE LISTING (42 sequences)

SEQ ID NO: 1 - RNA, 20 nt, synthetic construct
  source 1..20: mol_type = other RNA; note = A1
gggtgatgaagagaccaggg

SEQ ID NO: 2 - RNA, 20 nt, synthetic construct
  source 1..20: mol_type = other RNA; note = A2
ggactcactccatcacccgg

SEQ ID NO: 3 - RNA, 20 nt, synthetic construct
  source 1..20: mol_type = other RNA; note = A3
ggactccagatgctgcaggg

SEQ ID NO: 4 - RNA, 20 nt, synthetic construct
  source 1..20: mol_type = other RNA; note = A4
ggtgagtgagaacaagatcg

SEQ ID NO: 5 - RNA, 20 nt, synthetic construct
  source 1..20: mol_type = other RNA; note = A5
gggattcaggcagctcaacg

SEQ ID NO: 6 - RNA, 20 nt, synthetic construct
  source 1..20: mol_type = other RNA; note = A6
ggagggaggaaaaggccgtg

SEQ ID NO: 7 - RNA, 20 nt, synthetic construct
  source 1..20: mol_type = other RNA; note = A7
ggctgccttgagcgacacgg

SEQ ID NO: 8 - RNA, 20 nt, synthetic construct
  source 1..20: mol_type = other RNA; note = A8
gggagtttgcgtaagcaaag

SEQ ID NO: 9 - RNA, 20 nt, synthetic construct
  source 1..20: mol_type = other RNA; note = A9
ggacaagctgtcggaaacag

SEQ ID NO: 10 - RNA, 20 nt, synthetic construct
  source 1..20: mol_type = other RNA; note = A10
ggcctcggaagacacagctg

SEQ ID NO: 11 - RNA, 20 nt, synthetic construct
  source 1..20: mol_type = other RNA; note = A11
ggtcgctcaaggcagccctg

SEQ ID NO: 12 - RNA, 20 nt, synthetic construct
  source 1..20: mol_type = other RNA; note = A12
gggtggctgatggagcgaag

SEQ ID NO: 13 - RNA, 20 nt, synthetic construct
  source 1..20: mol_type = other RNA; note = A13
gggacaggtaggacccagca

SEQ ID NO: 14 - RNA, 20 nt, synthetic construct
  source 1..20: mol_type = other RNA; note = A14
gggttctgggacagactgcg

SEQ ID NO: 15 - RNA, 20 nt, synthetic construct
  source 1..20: mol_type = other RNA; note = A15
gggaacaagatcggggacga

SEQ ID NO: 16 - RNA, 20 nt, synthetic construct
  source 1..20: mol_type = other RNA; note = A16
ggtttaggtcccgaacagca

SEQ ID NO: 17 - RNA, 20 nt, synthetic construct
  source 1..20: mol_type = other RNA; note = A17
ggaagtggtagaggcacagg

SEQ ID NO: 18 - RNA, 20 nt, synthetic construct
  source 1..20: mol_type = other RNA; note = A18
ggagaagtggtagaggcaca

SEQ ID NO: 19 - RNA, 20 nt, synthetic construct
  source 1..20: mol_type = other RNA; note = A19
gggctgcctgaatctccctg

SEQ ID NO: 20 - RNA, 20 nt, synthetic construct
  source 1..20: mol_type = other RNA; note = A20
ggtctgtgtcgggttctggg

SEQ ID NO: 21 - RNA, 18 nt, synthetic construct
  source 1..18: mol_type = other RNA; note = A4-1
tgagtgagaacaagatcg

SEQ ID NO: 22 - RNA, 20 nt, synthetic construct
  source 1..20: mol_type = other RNA; note = A4-2
ctgagtgagaacaagatcgg

SEQ ID NO: 23 - RNA, 19 nt, synthetic construct
  source 1..19: mol_type = other RNA; note = A11-1
gtcgctcaaggcagccctg

SEQ ID NO: 24 - RNA, 20 nt, synthetic construct
  source 1..20: mol_type = other RNA; note = A11-2
gtcgctcaaggcagccctgt

SEQ ID NO: 25 - RNA, 18 nt, synthetic construct
  source 1..18: mol_type = other RNA; note = A15-1
gaacaagatcggggacga

SEQ ID NO: 26 - RNA, 20 nt, synthetic construct
  source 1..20: mol_type = other RNA; note = A15-2
gagaacaagatcggggacga

SEQ ID NO: 27 - RNA, 20 nt, synthetic construct
  source 1..20: mol_type = other RNA; note = TRAC sgRNA
agagtctctcagctggtaca

SEQ ID NO: 28 - protein, 107 aa, synthetic construct
  source 1..107: note = anti-CD19 VL
DIQMTQTTSSLSASLGDRVTISCRASQDISKYLNWYQQKPDGTVKLLIYHTSRLHSGVPSRFSGSGSGTDYSLTISNLEQEDIATYFCQQGNTLPYTFGGGTKLEIT

SEQ ID NO: 29 - protein, 120 aa, synthetic construct
  source 1..120: note = anti-CD19 VH
EVKLQESGPGLVAPSQSLSVTCTVSGVSLPDYGVSWIRQPPRKGLEWLGVIWGSETTYYNSALKSRLTIIKDNSKSQVFLKMNSLQTDDTAIYYCAKHYYYGGSYAMDYWGQGTSVTVSS

SEQ ID NO: 30 - protein, 242 aa, synthetic construct
  source 1..242: note = anti-CD19 scFv
DIQMTQTTSSLSASLGDRVTISCRASQDISKYLNWYQQKPDGTVKLLIYHTSRLHSGVPSRFSGSGSGTDYSLTISNLEQEDIATYFCQQGNTLPYTFGGGTKLEITGGGGSGGGGSGGGGSEVKLQESGPGLVAPSQSLSVTCTVSGVSLPDYGVSWIRQPPRKGLEWLGVIWGSETTYYNSALKSRLTIIKDNSKSQVFLKMNSLQTDDTAIYYCAKHYYYGGSYAMDYWGQGTSVTVSS

SEQ ID NO: 31 - protein, 25 aa, synthetic construct
  source 1..25: note = CD8alpha transmembrane domain
IYIWAPLAGTCGVLLLSLVITLYCK

SEQ ID NO: 32 - DNA, 75 bp, synthetic construct
  source 1..75: mol_type = other DNA; note = CD8alpha transmembrane domain
atctacatctgggcgcccttggccgggacttgtggggtccttctcctgtcactggttatcaccctttactgcaaa

SEQ ID NO: 33 - protein, 45 aa, synthetic construct
  source 1..45: note = CD8alpha hinge region
TTTPAPRPPTPAPTIASQPLSLRPEACRPAAGGAVHTRGLDFACD

SEQ ID NO: 34 - DNA, 135 bp, synthetic construct
  source 1..135: mol_type = other DNA; note = CD8alpha hinge region
accacgacgccagcgccgcgaccaccaacaccggcgcccaccatcgcgtcgcagcccctgtccctgcgcccagaggcgtgccggccagcggcggggggcgcagtgcacacgagggggctggacttcgcctgtgat

SEQ ID NO: 35 - protein, 113 aa, synthetic construct
  source 1..113: note = CD3zeta primary signaling domain
LRVKFSRSADAPAYQQGQNQLYNELNLGRREEYDVLDKRRGRDPEMGGKPRRKNPQEGLYNELQKDKMAEAYSEIGMKGERRRGKGHDGLYQGLSTATKDTYDALHMQALPPR

SEQ ID NO: 36 - DNA, 339 bp, synthetic construct
  source 1..339: mol_type = other DNA; note = CD3zeta primary signaling domain
ctgagagtgaagttcagcaggagcgcagacgcccccgcgtaccagcagggccagaaccagctctataacgagctcaatctaggacgaagagaggagtacgatgttttggacaagagacgtggccgggaccctgagatggggggaaagccgagaaggaagaaccctcaggaaggcctgtacaatgaactgcagaaagataagatggcggaggcctacagtgagattgggatgaaaggcgagcgccggaggggcaaggggcacgatggcctttaccagggtctcagtacagccaccaaggacacctacgacgcccttcacatgcaggccctgccccctcgc

SEQ ID NO: 37 - protein, 114 aa, synthetic construct
  source 1..114: note = CD3zeta primary signaling domain
LRVKFSRSADAPAYQQGQNQLFNELNLGRREEFDVLDKRRGRDPEMGGKPQRRKNPQEGLYNELQKDKMAEAYSEIGMKGERRRGKGHDGLFQGLSTATKDTFDALHMQALPPR

SEQ ID NO: 38 - DNA, 342 bp, synthetic construct
  source 1..342: mol_type = other DNA; note = CD3zeta primary signaling domain
ctgagagtgaagttcagcaggagcgcagacgcccccgcgtaccagcagggccagaaccagctctttaacgagctcaatctaggacgaagagaggagttcgatgttttggacaagagacgtggccgggaccctgagatggggggaaagccgcagagaaggaagaaccctcaggaaggcctgtacaatgaactgcagaaagataagatggcggaggcctacagtgagattgggatgaaaggcgagcgccggaggggcaaggggcacgatggccttttccagggtctcagtacagccaccaaggacacctttgacgcccttcacatgcaggccctgccccctcgc

SEQ ID NO: 39 - protein, 40 aa, synthetic construct
  source 1..40: note = 4-1BB costimulatory domain
RGRKKLLYIFKQPFMRPVQTTQEEDGCSCRFPEEEEGGCE

SEQ ID NO: 40 - DNA, 120 bp, synthetic construct
  source 1..120: mol_type = other DNA; note = 4-1BB costimulatory domain
cggggcagaaagaaactcctgtatatattcaaacaaccatttatgagaccagtacaaactactcaagaggaagatggctgtagctgccgatttccagaagaagaagaaggaggatgtgaa

SEQ ID NO: 41 - protein, 21 aa, synthetic construct
  source 1..21: note = CD8alpha signal peptide
MALPVTALLLPLALLLHAARP

SEQ ID NO: 42 - DNA, 63 bp, synthetic construct
  source 1..63: mol_type = other DNA; note = CD8alpha signal peptide
atggccttaccagtgaccgccttgctcctgccgctggccttgctgctccacgccgccaggccg